European Patent Specification EP 3 468 590 B1, published January 1, 2025. Title: NUCLEIC ACIDS ENCODING ZIKA VIRUS-LIKE PARTICLES AND THEIR USE IN ZIKA VIRUS VACCINES AND DIAGNOSTIC ASSAYS. Applicant: THE UNITED STATES OF AMERICA, AS REPRESENTED BY THE SECRETARY, DEPARTMENT OF HEALTH AND HUMAN SERVICES. The sequence listing filed with the application follows.

SEQUENCE LISTING (29 sequences)

SEQ ID NO: 1 - DNA, 5703 bp, Artificial Sequence
  Plasmid construct pEZMRprME1-8
ttcctgcgttatcccctgattctgtggataaccgtattaccgctagcatggatctcggggacgtctaactactaagcgagagtagggaactgccaggcatcaaataaaacgaaaggctcagtcggaagactgggcctttcgttttatctgttgtttgtcggtgaacgctctcctgagtaggacaaatccgccgggagcggatttgaacgttgtgaagcaacggcccggagggtggcgggcaggacgcccgccataaactgccaggcatcaaactaagcagaaggccatcctgacggatggcctttttgcgtttctacaaactcttcctgttagttagttacttaagctcgggccccaaataatgattttatttaactttgtacaaaaaagcaggcttcgaaggagatagaaccaattctctaaggaaatacttaaccatggtcgactggatccggtaccgaattcgtcgactagcccatatatggagttccgcgttacataacttacggtaaatggcccgcctggctgaccgcccaacgacccccgcccattgacgtcaataatgacgtatgttcccatagtaacgccaatagggactttccattgacgtcaatgggtggagtatttacggtaaactgcccacttggcagtacatcaagtgtatcatatgccaagtacgccccctattgacgtcaatgacggtaaatggcccgcctggcattatgcccagtacatgaccttatgggactttcctacttggcagtacatctacgtattagtcatcgctattaccatggtgatgcggttttggcagtacatcaatgggcgtggatagcggtttgactcacggggatttccaagtctccaccccattgacgtcaatgggagtttgttttggcaccaaaatcaacgggactttccaaaatgtcgtaacaactccgccccattgacgcaaatgggcggtaggcgtgtacggtgggaggtctatataagcagagctctctggctaactagagaacccactgcttactggcttatcgaaattaatacgactcactatagggagacccaagctggctagcgtttaaacttaagcttggtaccgccgccgccatgggcaagaggtccgccggctcaatcatgtggctcgcgagcttggcagttgtcatagctggtacaagcgctgcagagatcactagacgcgggagtgcatactacatgtacttggataggagcgatgccgggaaggccatttcgtttgctaccacattgggagtgaacaagtgccacgtacagatcatggacctcgggcacatgtgtgacgccaccatgagttatgagtgccctatgctggatgagggagtggaaccagatgatgtcgattgctggtgcaacacgacatcaacttgggttgtgtacggaacctgtcatcacaaaaaaggtgaggcacggcgatctagaagagccgtgacgctcccttctcactctacgaggaagttgcaaacgcggtcgcagacctggttagaatcaagagaatacacgaagcacttgatcaaggttgaaaactggatattcaggaaccccgggtttgcgctagtggccgttgccattgcctggcttttgggaagctcgacgagccaaaaagtcatatacttggtcatgatactgctgattgccccggcatacagtatcaggtgcattggagtcagcaatagagacttcgtggagggcatgtcaggtgggacctgggttgatgttgtcttggaacatggaggctgcgttaccgtgatggcacaggacaagccaacagttgacatagagttggtcacgacgacggttagtaacatggccgaggtaagatcctattgctacgaggcatcgatatcggacatggcttcggacagtcgttgcccaacacaaggtgaagcctaccttgacaagcaatcagacactcaatatgtctgcaaaagaacattagtggacagaggttggggaaacggttgtggactttttggcaaagggagcttggtgacatgtgccaagtttacgtgttctaagaagatgaccgggaagagcattcaaccggaaaatctggagtatcggataatgctatcagtgcatggctcccagcatagcgggatgattgtcaatgatacaggatatgaaactgacgaaaatagagcgaaagtcgaggttacgcctaattcaccaagagcggaagcaaccttgggaggctttggaagcttaggacttgactgtgaaccaaggacaggccttgacttttcagatctgtattacctgaccatgaacaataagcattggttggtgcacaaagagtggtttcatgacatcccattgccttggcatgctggggcagacaccggaactccacactggaacaacaaagaggcattggtagaattcaaggatgcccacgccaagaggcaaaccgtcgtcgttctggggagccaggaaggagccgttcacacggctctcgctggagctctagaggctgagatggatggtgcaaagggaaagctgttctctggccatttgaaatgccgcctaaaaatggacaagcttagattgaagggcgtgtcatattccttgtgcactgcggcattcacattcaccaaggtcccagctgaaacactgcatggaacagtcacagtggaggtgcagtatgcagggacagatggaccctgcaagatcccagtccagatggcggtggacatgcagaccctgaccccagttggagggctgataaccgccaaccccgtgattactgaaagcactgagaactcaaagatgatgttggagcttgacccaccatttggggattcttacattgtcataggagttggggacaagaaaatcacccaccactggcataggagtggtagcaccatcggaaaggcatttgaggccactgtgagaggcgccaagagaatggcagtcctgggggatacagcctgggacttcggatcagtcgggggtgtgttcaactcactgggtaagggcattcaccagatttttggagcagccttcaaatcactgtttggaggaatgtcctggttctcacagatcctcataggcacgctgctagtgtggttaggtttgaacacaaagaatggatctatctccctcacatgcttggccctggggggagtgatgatcttcctctccacggctgtttctgcttgagcggccgctcgagtctagagggcccgtttaaacccgctgatcagcctcgactgtgccttctagttgccagccatctgttgtttgcccctcccccgtgccttccttgaccctggaaggtgccactcccactgtcctttcctaataaaatgaggaaattgcatcgcattgtctgagtaggtgtcattctattctggggggtggggtggggcaggacagcaagggggaggattgggaagacaatagcaggcatgctggggatgcggtgggctctatggcttctactgggcggttttatggacagcaagcgaaccggaattgccagctggggcgccctctggtaaggtgatatctagacccagctttcttgtacaaagttggcattataagaaagcattgcttatcaatttgttgcaacgaacaggtcactatcagtcaaaataaaatcattatttgccatccagctgcagctctggcccgtgtctcaaaatctctgatgttacattgcacaagataaaaatatatcatcatgaacaataaaactgtctgcttacataaacagtaatacaaggggtgttatgagccatattcaacgggaaacgtcgaggccgcgattaaattccaacatggatgctgatttatatgggtataaatgggctcgcgataatgtcgggcaatcaggtgcgacaatctatcgcttgtatgggaagcccgatgcgccagagttgtttctgaaacatggcaaaggtagcgttgccaatgatgttacagatgagatggtcagactaaactggctgacggaatttatgcctcttccgaccatcaagcattttatccgtactcctgatgatgcatggttactcaccactgcgatccccggaaaaacagcattccaggtattagaagaatatcctgattcaggtgaaaatattgttgatgcgctggcagtgttcctgcgccggttgcattcgattcctgtttgtaattgtccttttaacagcgatcgcgtatttcgtctcgctcaggcgcaatcacgaatgaataacggtttggttgatgcgagtgattttgatgacgagcgtaatggctggcctgttgaacaagtctggaaagaaatgcataaacttttgccattctcaccggattcagtcgtcactcatggtgatttctcacttgataaccttatttttgacgaggggaaattaataggttgtattgatgttggacgagtcggaatcgcagaccgataccaggatcttgccatcctatggaactgcctcggtgagttttctccttcattacagaaacggctttttcaaaaatatggtattgataatcctgatatgaataaattgcagtttcatttgatgctcgatgagtttttctaatcagaattggttaattggttgtaacattattcagattgggccccgttccactgagcgtcagaccccgtagaaaagatcaaaggatcttcttgagatcctttttttctgcgcgtaatctgctgcttgcaaacaaaaaaaccaccgctaccagcggtggtttgtttgccggatcaagagctaccaactctttttccgaaggtaactggcttcagcagagcgcagataccaaatactgttcttctagtgtagccgtagttaggccaccacttcaagaactctgtagcaccgcctacatacctcgctctgctaatcctgttaccagtggctgctgccagtggcgataagtcgtgtcttaccgggttggactcaagacgatagttaccggataaggcgcagcggtcgggctgaacggggggttcgtgcacacagcccagcttggagcgaacgacctacaccgaactgagatacctacagcgtgagctatgagaaagcgccacgcttcccgaagggagaaaggcggacaggtatccggtaagcggcagggtcggaacaggagagcgcacgagggagcttccagggggaaacgcctggtatctttatagtcctgtcgggtttcgccacctctgacttgagcgtcgatttttgtgatgctcgtcaggggggcggagcctatggaaaaacgccagcaacgcggcctttttacggttcctggccttttgctggccttttgctcacatgttctttcctgcgttatcccctgattctgtggataaccgtattaccgctagcatggatctcggggacgtctaactactaagcgagagtagggaactgccaggcatcaaataaaacgaaaggctcagtcggaagactgggcctttcgttttatctgttgtttgtcggtgaacgctctcctgagtaggacaaatccgccgggagcggatttgaacgttgtgaagcaacggcccggagggtggcgggcaggacgcccgccataaactgccaggcatcaaactaagcagaaggccatcctgacggatggcctttttgcgtttctacaaactcttcctgttagttagttacttaagctcgggccccaaataatgattttatt

SEQ ID NO: 2 - DNA, 5712 bp, Artificial Sequence
  Plasmid construct pEBZHu8
ttcctgcgttatcccctgattctgtggataaccgtattaccgctagcatggatctcggggacgtctaactactaagcgagagtagggaactgccaggcatcaaataaaacgaaaggctcagtcggaagactgggcctttcgttttatctgttgtttgtcggtgaacgctctcctgagtaggacaaatccgccgggagcggatttgaacgttgtgaagcaacggcccggagggtggcgggcaggacgcccgccataaactgccaggcatcaaactaagcagaaggccatcctgacggatggcctttttgcgtttctacaaactcttcctgttagttagttacttaagctcgggccccaaataatgattttatttaactttgtacaaaaaagcaggcttcgaaggagatagaaccaattctctaaggaaatacttaaccatggtcgactggatccggtaccgaattcgtcgactagcccatatatggagttccgcgttacataacttacggtaaatggcccgcctggctgaccgcccaacgacccccgcccattgacgtcaataatgacgtatgttcccatagtaacgccaatagggactttccattgacgtcaatgggtggagtatttacggtaaactgcccacttggcagtacatcaagtgtatcatatgccaagtacgccccctattgacgtcaatgacggtaaatggcccgcctggcattatgcccagtacatgaccttatgggactttcctacttggcagtacatctacgtattagtcatcgctattaccatggtgatgcggttttggcagtacatcaatgggcgtggatagcggtttgactcacggggatttccaagtctccaccccattgacgtcaatgggagtttgttttggcaccaaaatcaacgggactttccaaaatgtcgtaacaactccgccccattgacgcaaatgggcggtaggcgtgtacggtgggaggtctatataagcagagctctctggctaactagagaacccactgcttactggcttatcgaaattaatacgactcactatagggagacccaagctggctagcgtttaaacttaagcttggtaccgccgccgccatgggcaagaggtccgccggctcaatcatgtggctcgcgagcttggcagttgtcatagctggtacaagcgctgccgtggaagtgaccagaagaggcagcgcctactacatgtacctggaccggaacgatgccggcgaggccatcagctttccaaccaccctgggcatgaacaagtgctacatccagatcatggacctgggccacatgtgcgacgccaccatgagctacgagtgccccatgctggacgagggcgtggaacccgacgatgtggactgctggtgcaacaccaccagcacctgggtggtgtacggcacctgtcaccacaagaagggcgaagccagacggtccagacgggccgtgacactgcctagccacagcaccagaaagctgcagacccggtcccagacctggctggaaagcagagagtacaccaagcacctgatccgggtggaaaactggatcttccggaaccccggctttgccctggccgctgctgctattgcttggctgctgggcagcagcacctcccagaaagtgatctacctcgtgatgatcctgctgatcgcccctgcctacagcatccggtgtatcggcgtgtccaaccgggacttcgtggaaggcatgagcggcggcacatgggtggacatcgtgctggaacacggcggctgcgtgacagtgatggcccaggataagcccaccgtggacattgagctcgtgaccaccaccgtgtccaatatggccgaagtgcggagctactgctacgaggccagcatcagcgacatggccagcgacagcagatgccccacacagggcgaggcttacctggacaagcagtccgacacccagtacgtgtgcaagcggaccctggtggatagaggctggggcaatggctgcggcctgtttggcaagggcagcctcgtgacctgcgccaagttcgcctgcagcaagaagatgaccggcaagagcatccagcccgagaacctggaataccggatcatgctgagcgtgcacggcagccagcactccggcatgatcgtgaacgacaccggccacgagacagacgagaaccgggccaaggtggaaatcacccccaacagccctagagccgaggccacactgggcggctttggatctctgggcctggactgcgagcctagaaccggcctggatttcagcgacctgtactacctgaccatgaacaacaagcactggctggtgcacaaagagtggttccacgacatccccctgccctggcatgccggcgctgatacaggcacaccccactggaacaacaaagaggctctggtggagttcaaggacgcccacgccaagaggcagaccgtggtggtgctgggatctcaggaaggcgccgtgcatacagctctggctggcgccctggaagccgaaatggatggcgctaagggcagactgtccagcggccacctgaagtgccggctgaagatggacaagctgcggctgaagggcgtgtcctacagcctgtgtaccgccgccttcaccttcaccaagatccccgccgagacactgcacggcaccgtgactgtggaagtgcagtacgccggcaccgacggcccttgtaaagtgcctgctcagatggccgtggatatgcagaccctgacccctgtgggcaggctgatcaccgccaaccctgtgatcaccgagagcaccgagaacagcaagatgatgctggaactggacccccccttcggcgactcctacatcgtgatcggcgtgggagagaagaagatcacccaccactggcacagaagcggcagcaccatcggcaaagccttcgaagccacagtgcggggagccaagagaatggccgtgctgggagataccgcctgggactttggctctgtgggcggagccctgaactctctgggcaagggaatccaccagatcttcggagccgcctttaagagcctgttcggcggcatgagctggttcagccagatcctgatcggcaccctgctgatgtggctgggcctgaacaccaagaacggcagcatctccctgatgtgcctggctctgggaggcgtgctgatcttcctgagcacagccgtgtctgccgacgtgtgagcggccgctcgagtctagagggcccgtttaaacccgctgatcagcctcgactgtgccttctagttgccagccatctgttgtttgcccctcccccgtgccttccttgaccctggaaggtgccactcccactgtcctttcctaataaaatgaggaaattgcatcgcattgtctgagtaggtgtcattctattctggggggtggggtggggcaggacagcaagggggaggattgggaagacaatagcaggcatgctggggatgcggtgggctctatggcttctactgggcggttttatggacagcaagcgaaccggaattgccagctggggcgccctctggtaaggtgatatctagacccagctttcttgtacaaagttggcattataagaaagcattgcttatcaatttgttgcaacgaacaggtcactatcagtcaaaataaaatcattatttgccatccagctgcagctctggcccgtgtctcaaaatctctgatgttacattgcacaagataaaaatatatcatcatgaacaataaaactgtctgcttacataaacagtaatacaaggggtgttatgagccatattcaacgggaaacgtcgaggccgcgattaaattccaacatggatgctgatttatatgggtataaatgggctcgcgataatgtcgggcaatcaggtgcgacaatctatcgcttgtatgggaagcccgatgcgccagagttgtttctgaaacatggcaaaggtagcgttgccaatgatgttacagatgagatggtcagactaaactggctgacggaatttatgcctcttccgaccatcaagcattttatccgtactcctgatgatgcatggttactcaccactgcgatccccggaaaaacagcattccaggtattagaagaatatcctgattcaggtgaaaatattgttgatgcgctggcagtgttcctgcgccggttgcattcgattcctgtttgtaattgtccttttaacagcgatcgcgtatttcgtctcgctcaggcgcaatcacgaatgaataacggtttggttgatgcgagtgattttgatgacgagcgtaatggctggcctgttgaacaagtctggaaagaaatgcataaacttttgccattctcaccggattcagtcgtcactcatggtgatttctcacttgataaccttatttttgacgaggggaaattaataggttgtattgatgttggacgagtcggaatcgcagaccgataccaggatcttgccatcctatggaactgcctcggtgagttttctccttcattacagaaacggctttttcaaaaatatggtattgataatcctgatatgaataaattgcagtttcatttgatgctcgatgagtttttctaatcagaattggttaattggttgtaacattattcagattgggccccgttccactgagcgtcagaccccgtagaaaagatcaaaggatcttcttgagatcctttttttctgcgcgtaatctgctgcttgcaaacaaaaaaaccaccgctaccagcggtggtttgtttgccggatcaagagctaccaactctttttccgaaggtaactggcttcagcagagcgcagataccaaatactgttcttctagtgtagccgtagttaggccaccacttcaagaactctgtagcaccgcctacatacctcgctctgctaatcctgttaccagtggctgctgccagtggcgataagtcgtgtcttaccgggttggactcaagacgatagttaccggataaggcgcagcggtcgggctgaacggggggttcgtgcacacagcccagcttggagcgaacgacctacaccgaactgagatacctacagcgtgagctatgagaaagcgccacgcttcccgaagggagaaaggcggacaggtatccggtaagcggcagggtcggaacaggagagcgcacgagggagcttccagggggaaacgcctggtatctttatagtcctgtcgggtttcgccacctctgacttgagcgtcgatttttgtgatgctcgtcaggggggcggagcctatggaaaaacgccagcaacgcggcctttttacggttcctggccttttgctggccttttgctcacatgttctttcctgcgttatcccctgattctgtggataaccgtattaccgctagcatggatctcggggacgtctaactactaagcgagagtagggaactgccaggcatcaaataaaacgaaaggctcagtcggaagactgggcctttcgttttatctgttgtttgtcggtgaacgctctcctgagtaggacaaatccgccgggagcggatttgaacgttgtgaagcaacggcccggagggtggcgggcaggacgcccgccataaactgccaggcatcaaactaagcagaaggccatcctgacggatggcctttttgcgtttctacaaactcttcctgttagttagttacttaagctcgggccccaaataatgattttatt

SEQ ID NO: 3 - DNA, 5709 bp, Artificial Sequence
  Plasmid construct pEBZHu2-3
ttcctgcgttatcccctgattctgtggataaccgtattaccgctagcatggatctcggggacgtctaactactaagcgagagtagggaactgccaggcatcaaataaaacgaaaggctcagtcggaagactgggcctttcgttttatctgttgtttgtcggtgaacgctctcctgagtaggacaaatccgccgggagcggatttgaacgttgtgaagcaacggcccggagggtggcgggcaggacgcccgccataaactgccaggcatcaaactaagcagaaggccatcctgacggatggcctttttgcgtttctacaaactcttcctgttagttagttacttaagctcgggccccaaataatgattttatttaactttgtacaaaaaagcaggcttcgaaggagatagaaccaattctctaaggaaatacttaaccatggtcgactggatccggtaccgaattcgtcgactagcccatatatggagttccgcgttacataacttacggtaaatggcccgcctggctgaccgcccaacgacccccgcccattgacgtcaataatgacgtatgttcccatagtaacgccaatagggactttccattgacgtcaatgggtggagtatttacggtaaactgcccacttggcagtacatcaagtgtatcatatgccaagtacgccccctattgacgtcaatgacggtaaatggcccgcctggcattatgcccagtacatgaccttatgggactttcctacttggcagtacatctacgtattagtcatcgctattaccatggtgatgcggttttggcagtacatcaatgggcgtggatagcggtttgactcacggggatttccaagtctccaccccattgacgtcaatgggagtttgttttggcaccaaaatcaacgggactttccaaaatgtcgtaacaactccgccccattgacgcaaatgggcggtaggcgtgtacggtgggaggtctatataagcagagctctctggctaactagagaacccactgcttactggcttatcgaaattaatacgactcactatagggagacccaagctggctagcgtttaaacttaagcttggtaccgccgccgccatgggcaagaggtccgccggctcaatcatgtggctcgcgagcttggcagttgtcatagctggtacaagcgccgtggaagtgaccagaagaggcagcgcctactacatgtacctggaccggaacgatgccggcgaggccatcagctttccaaccaccctgggcatgaacaagtgctacatccagatcatggacctgggccacatgtgcgacgccaccatgagctacgagtgccccatgctggacgagggcgtggaacccgacgatgtggactgctggtgcaacaccaccagcacctgggtggtgtacggcacctgtcaccacaagaagggcgaagccagacggtccagacgggccgtgacactgcctagccacagcaccagaaagctgcagacccggtcccagacctggctggaaagcagagagtacaccaagcacctgatccgggtggaaaactggatcttccggaaccccggctttgccctggccgctgctgctattgcttggctgctgggcagcagcacctcccagaaagtgatctacctcgtgatgatcctgctgatcgcccctgcctacagcatccggtgtatcggcgtgtccaaccgggacttcgtggaaggcatgagcggcggcacatgggtggacatcgtgctggaacacggcggctgcgtgacagtgatggcccaggataagcccaccgtggacattgagctcgtgaccaccaccgtgtccaatatggccgaagtgcggagctactgctacgaggccagcatcagcgacatggccagcgacagcagatgccccacacagggcgaggcttacctggacaagcagtccgacacccagtacgtgtgcaagcggaccctggtggatagaggctggggcaatggctgcggcctgtttggcaagggcagcctcgtgacctgcgccaagttcgcctgcagcaagaagatgaccggcaagagcatccagcccgagaacctggaataccggatcatgctgagcgtgcacggcagccagcactccggcatgatcgtgaacgacaccggccacgagacagacgagaaccgggccaaggtggaaatcacccccaacagccctagagccgaggccacactgggcggctttggatctctgggcctggactgcgagcctagaaccggcctggatttcagcgacctgtactacctgaccatgaacaacaagcactggctggtgcacaaagagtggttccacgacatccccctgccctggcatgccggcgctgatacaggcacaccccactggaacaacaaagaggctctggtggagttcaaggacgcccacgccaagaggcagaccgtggtggtgctgggatctcaggaaggcgccgtgcatacagctctggctggcgccctggaagccgaaatggatggcgctaagggcagactgtccagcggccacctgaagtgccggctgaagatggacaagctgcggctgaagggcgtgtcctacagcctgtgtaccgccgccttcaccttcaccaagatccccgccgagacactgcacggcaccgtgactgtggaagtgcagtacgccggcaccgacggcccttgtaaagtgcctgctcagatggccgtggatatgcagaccctgacccctgtgggcaggctgatcaccgccaaccctgtgatcaccgagagcaccgagaacagcaagatgatgctggaactggacccccccttcggcgactcctacatcgtgatcggcgtgggagagaagaagatcacccaccactggcacagaagcggcagcaccatcggcaaagccttcgaagccacagtgcggggagccaagagaatggccgtgctgggagataccgcctgggactttggctctgtgggcggagccctgaactctctgggcaagggaatccaccagatcttcggagccgcctttaagagcctgttcggcggcatgagctggttcagccagatcctgatcggcaccctgctgatgtggctgggcctgaacaccaagaacggcagcatctccctgatgtgcctggctctgggaggcgtgctgatcttcctgagcacagccgtgtctgccgacgtgtgagcggccgctcgagtctagagggcccgtttaaacccgctgatcagcctcgactgtgccttctagttgccagccatctgttgtttgcccctcccccgtgccttccttgaccctggaaggtgccactcccactgtcctttcctaataaaatgaggaaattgcatcgcattgtctgagtaggtgtcattctattctggggggtggggtggggcaggacagcaagggggaggattgggaagacaatagcaggcatgctggggatgcggtgggctctatggcttctactgggcggttttatggacagcaagcgaaccggaattgccagctggggcgccctctggtaaggtgatatctagacccagctttcttgtacaaagttggcattataagaaagcattgcttatcaatttgttgcaacgaacaggtcactatcagtcaaaataaaatcattatttgccatccagctgcagctctggcccgtgtctcaaaatctctgatgttacattgcacaagataaaaatatatcatcatgaacaataaaactgtctgcttacataaacagtaatacaaggggtgttatgagccatattcaacgggaaacgtcgaggccgcgattaaattccaacatggatgctgatttatatgggtataaatgggctcgcgataatgtcgggcaatcaggtgcgacaatctatcgcttgtatgggaagcccgatgcgccagagttgtttctgaaacatggcaaaggtagcgttgccaatgatgttacagatgagatggtcagactaaactggctgacggaatttatgcctcttccgaccatcaagcattttatccgtactcctgatgatgcatggttactcaccactgcgatccccggaaaaacagcattccaggtattagaagaatatcctgattcaggtgaaaatattgttgatgcgctggcagtgttcctgcgccggttgcattcgattcctgtttgtaattgtccttttaacagcgatcgcgtatttcgtctcgctcaggcgcaatcacgaatgaataacggtttggttgatgcgagtgattttgatgacgagcgtaatggctggcctgttgaacaagtctggaaagaaatgcataaacttttgccattctcaccggattcagtcgtcactcatggtgatttctcacttgataaccttatttttgacgaggggaaattaataggttgtattgatgttggacgagtcggaatcgcagaccgataccaggatcttgccatcctatggaactgcctcggtgagttttctccttcattacagaaacggctttttcaaaaatatggtattgataatcctgatatgaataaattgcagtttcatttgatgctcgatgagtttttctaatcagaattggttaattggttgtaacattattcagattgggccccgttccactgagcgtcagaccccgtagaaaagatcaaaggatcttcttgagatcctttttttctgcgcgtaatctgctgcttgcaaacaaaaaaaccaccgctaccagcggtggtttgtttgccggatcaagagctaccaactctttttccgaaggtaactggcttcagcagagcgcagataccaaatactgttcttctagtgtagccgtagttaggccaccacttcaagaactctgtagcaccgcctacatacctcgctctgctaatcctgttaccagtggctgctgccagtggcgataagtcgtgtcttaccgggttggactcaagacgatagttaccggataaggcgcagcggtcgggctgaacggggggttcgtgcacacagcccagcttggagcgaacgacctacaccgaactgagatacctacagcgtgagctatgagaaagcgccacgcttcccgaagggagaaaggcggacaggtatccggtaagcggcagggtcggaacaggagagcgcacgagggagcttccagggggaaacgcctggtatctttatagtcctgtcgggtttcgccacctctgacttgagcgtcgatttttgtgatgctcgtcaggggggcggagcctatggaaaaacgccagcaacgcggcctttttacggttcctggccttttgctggccttttgctcacatgttctttcctgcgttatcccctgattctgtggataaccgtattaccgctagcatggatctcggggacgtctaactactaagcgagagtagggaactgccaggcatcaaataaaacgaaaggctcagtcggaagactgggcctttcgttttatctgttgtttgtcggtgaacgctctcctgagtaggacaaatccgccgggagcggatttgaacgttgtgaagcaacggcccggagggtggcgggcaggacgcccgccataaactgccaggcatcaaactaagcagaaggccatcctgacggatggcctttttgcgtttctacaaactcttcctgttagttagttacttaagctcgggccccaaataatgattttatt

SEQ ID NO: 4 - protein, 24 aa, Artificial Sequence
  Modified JEV signal sequence
MGKRSAGSIMWLASLAVVIAGTSA

SEQ ID NO: 5 - protein, 672 aa, Artificial Sequence
  prME protein expressed by pEZMRprME1-8
AEITRRGSAYYMYLDRSDAGKAISFATTLGVNKCHVQIMDLGHMCDATMSYECPMLDEGVEPDDVDCWCNTTSTWVVYGTCHHKKGEARRSRRAVTLPSHSTRKLQTRSQTWLESREYTKHLIKVENWIFRNPGFALVAVAIAWLLGSSTSQKVIYLVMILLIAPAYSIRCIGVSNRDFVEGMSGGTWVDVVLEHGGCVTVMAQDKPTVDIELVTTTVSNMAEVRSYCYEASISDMASDSRCPTQGEAYLDKQSDTQYVCKRTLVDRGWGNGCGLFGKGSLVTCAKFTCSKKMTGKSIQPENLEYRIMLSVHGSQHSGMIVNDTGYETDENRAKVEVTPNSPRAEATLGGFGSLGLDCEPRTGLDFSDLYYLTMNNKHWLVHKEWFHDIPLPWHAGADTGTPHWNNKEALVEFKDAHAKRQTVVVLGSQEGAVHTALAGALEAEMDGAKGKLFSGHLKCRLKMDKLRLKGVSYSLCTAAFTFTKVPAETLHGTVTVEVQYAGTDGPCKIPVQMAVDMQTLTPVGGLITANPVITESTENSKMMLELDPPFGDSYIVIGVGDKKITHHWHRSGSTIGKAFEATVRGAKRMAVLGDTAWDFGSVGGVFNSLGKGIHQIFGAAFKSLFGGMSWFSQILIGTLLVWLGLNTKNGSISLTCLALGGVMIFLSTAVSA

SEQ ID NO: 6 - protein, 675 aa, Artificial Sequence
  prME protein expressed by pEBZHu8
AVEVTRRGSAYYMYLDRNDAGEAISFPTTLGMNKCYIQIMDLGHMCDATMSYECPMLDEGVEPDDVDCWCNTTSTWVVYGTCHHKKGEARRSRRAVTLPSHSTRKLQTRSQTWLESREYTKHLIRVENWIFRNPGFALAAAAIAWLLGSSTSQKVIYLVMILLIAPAYSIRCIGVSNRDFVEGMSGGTWVDIVLEHGGCVTVMAQDKPTVDIELVTTTVSNMAEVRSYCYEASISDMASDSRCPTQGEAYLDKQSDTQYVCKRTLVDRGWGNGCGLFGKGSLVTCAKFACSKKMTGKSIQPENLEYRIMLSVHGSQHSGMIVNDTGHETDENRAKVEITPNSPRAEATLGGFGSLGLDCEPRTGLDFSDLYYLTMNNKHWLVHKEWFHDIPLPWHAGADTGTPHWNNKEALVEFKDAHAKRQTVVVLGSQEGAVHTALAGALEAEMDGAKGRLSSGHLKCRLKMDKLRLKGVSYSLCTAAFTFTKIPAETLHGTVTVEVQYAGTDGPCKVPAQMAVDMQTLTPVGRLITANPVITESTENSKMMLELDPPFGDSYIVIGVGEKKITHHWHRSGSTIGKAFEATVRGAKRMAVLGDTAWDFGSVGGALNSLGKGIHQIFGAAFKSLFGGMSWFSQILIGTLLMWLGLNTKNGSISLMCLALGGVLIFLSTAVSADV

SEQ ID NO: 7 - protein, 674 aa, Artificial Sequence
  prME protein expressed by pEBZHu2-3
VEVTRRGSAYYMYLDRNDAGEAISFPTTLGMNKCYIQIMDLGHMCDATMSYECPMLDEGVEPDDVDCWCNTTSTWVVYGTCHHKKGEARRSRRAVTLPSHSTRKLQTRSQTWLESREYTKHLIRVENWIFRNPGFALAAAAIAWLLGSSTSQKVIYLVMILLIAPAYSIRCIGVSNRDFVEGMSGGTWVDIVLEHGGCVTVMAQDKPTVDIELVTTTVSNMAEVRSYCYEASISDMASDSRCPTQGEAYLDKQSDTQYVCKRTLVDRGWGNGCGLFGKGSLVTCAKFACSKKMTGKSIQPENLEYRIMLSVHGSQHSGMIVNDTGHETDENRAKVEITPNSPRAEATLGGFGSLGLDCEPRTGLDFSDLYYLTMNNKHWLVHKEWFHDIPLPWHAGADTGTPHWNNKEALVEFKDAHAKRQTVVVLGSQEGAVHTALAGALEAEMDGAKGRLSSGHLKCRLKMDKLRLKGVSYSLCTAAFTFTKIPAETLHGTVTVEVQYAGTDGPCKVPAQMAVDMQTLTPVGRLITANPVITESTENSKMMLELDPPFGDSYIVIGVGEKKITHHWHRSGSTIGKAFEATVRGAKRMAVLGDTAWDFGSVGGALNSLGKGIHQIFGAAFKSLFGGMSWFSQILIGTLLMWLGLNTKNGSISLMCLALGGVLIFLSTAVSADV

SEQ ID NO: 8 - DNA, 13 bp, Artificial Sequence
  Kozak consensus sequence
gccgccgccatgg

SEQ ID NO: 9 - protein, 43 aa, Artificial Sequence
  Synthetic polypeptide
RKEKKRRGADTSIGIVGLLLTTAMAAEITRRGSAYYMYLDRSD

SEQ ID NO: 10 - protein, 36 aa, Artificial Sequence
  Synthetic polypeptide
GADTSIGIVGLLLTTAMAAEITRRGSAYYMYLDRSD

SEQ ID NO: 11 - protein, 36 aa, Artificial Sequence
  Synthetic polypeptide
GADTSIGIVGLLLTTAMAAEVTRRGSAYYMYLDRND

SEQ ID NO: 12 - protein, 43 aa, Artificial Sequence
  Synthetic polypeptide
RKEKKRRGADTSVGIVGLLLTTAMAAEVTRRGSAYYMYLDRND

SEQ ID NO: 13 - protein, 36 aa, Artificial Sequence
  Synthetic polypeptide
GADTSVGIVGLLLTTAMAAEVTRRGSAYYMYLDRND

SEQ ID NO: 14 - protein, 42 aa, Artificial Sequence
  Synthetic polypeptide
MGKRSAGSIMWLASLAVVIAGTSAAEITRRGSAYYMYLDRSD

SEQ ID NO: 15 - protein, 42 aa, Artificial Sequence
  Synthetic polypeptide
MGKRSAGSIMWLASLAVVIAGTSAAEVTRRGSAYYMYLDRND

SEQ ID NO: 16 - protein, 41 aa, Artificial Sequence
  Synthetic polypeptide
MGKRSAGSIMWLASLAVVIAGTSAEVTRRGSAYYMYLDRND

SEQ ID NO: 17 - protein, 41 aa, Artificial Sequence
  Synthetic polypeptide
MGKRSAGSIMWLASLAVVIAGTSAAETRRGSAYYMYLDRND

SEQ ID NO: 18 - protein, 43 aa, Artificial Sequence
  Synthetic polypeptide
MGKRSAGSIMWLASLAVVIAGTSAAVEVTRRGSAYYMYLDRND

SEQ ID NO: 19 - protein, 42 aa, Artificial Sequence
  Synthetic polypeptide
MGKRSAGSIMWLASLAVVIAGTSAVEVTRRGSAYYMYLDRND

SEQ ID NO: 20 - DNA, 5328 bp, Artificial Sequence
  Plasmid construct pEZMRprME KD
ctttgtacaaaaaagcaggcttcgaaggagatagaaccaattctctaaggaaatacttaaccatggtcgactggatccggtaccgaattcgtcgactagcccatatatggagttccgcgttacataacttacggtaaatggcccgcctggctgaccgcccaacgacccccgcccattgacgtcaataatgacgtatgttcccatagtaacgccaatagggactttccattgacgtcaatgggtggagtatttacggtaaactgcccacttggcagtacatcaagtgtatcatatgccaagtacgccccctattgacgtcaatgacggtaaatggcccgcctggcattatgcccagtacatgaccttatgggactttcctacttggcagtacatctacgtattagtcatcgctattaccatggtgatgcggttttggcagtacatcaatgggcgtggatagcggtttgactcacggggatttccaagtctccaccccattgacgtcaatgggagtttgttttggcaccaaaatcaacgggactttccaaaatgtcgtaacaactccgccccattgacgcaaatgggcggtaggcgtgtacggtgggaggtctatataagcagagctctctggctaactagagaacccactgcttactggcttatcgaaattaatacgactcactatagggagacccaagctggctagcgtttaaacttaagcttggtaccgccgccgccatgggcaagaggtccgccggctcaatcatgtggctcgcgagcttggcagttgtcatagctggtacaagcgctgcagagatcactagacgcgggagtgcatactacatgtacttggataggagcgatgccgggaaggccatttcgtttgctaccacattgggagtgaacaagtgccacgtacagatcatggacctcgggcacatgtgtgacgccaccatgagttatgagtgccctatgctggatgagggagtggaaccagatgatgtcgattgctggtgcaacacgacatcaacttgggttgtgtacggaacctgtcatcacaaaaaaggtgaggcacggcgatctagaagagccgtgacgctcccttctcactctacgaggaagttgcaaacgcggtcgcagacctggttagaatcaagagaatacacgaagcacttgatcaaggttgaaaactggatattcaggaaccccgggtttgcgctagtggccgttgccattgcctggcttttgggaagctcgacgagccaaaaagtcatatacttggtcatgatactgctgattgccccggcatacagtatcaggtgcattggagtcagcaatagagacttcgtggagggcatgtcaggtgggacctgggttgatgttgtcttggaacatggaggctgcgttaccgtgatggcacaggacaagccaacagttgacatagagttggtcacgacgacggttagtaacatggccgaggtaagatcctattgctacgaggcatcgatatcggacatggcttcggacagtcgttgcccaacacaaggtgaagcctaccttgacaagcaatcagacactcaatatgtctgcaaaagaacattagtggacagaggttggggaaacggttgtaaggattttggcaaagggagcttggtgacatgtgccaagtttacgtgttctaagaagatgaccgggaagagcattcaaccggaaaatctggagtatcggataatgctatcagtgcatggctcccagcatagcgggatgattgtcaatgatacaggatatgaaactgacgaaaatagagcgaaagtcgaggttacgcctaattcaccaagagcggaagcaaccttgggaggctttggaagcttaggacttgactgtgaaccaaggacaggccttgacttttcagatctgtattacctgaccatgaacaataagcattggttggtgcacaaagagtggtttcatgacatcccattgccttggcatgctggggcagacaccggaactccacactggaacaacaaagaggcattggtagaattcaaggatgcccacgccaagaggcaaaccgtcgtcgttctggggagccaggaaggagccgttcacacggctctcgctggagctctagaggctgagatggatggtgcaaagggaaagctgttctctggccatttgaaatgccgcctaaaaatggacaagcttagattgaagggcgtgtcatattccttgtgcactgcggcattcacattcaccaaggtcccagctgaaacactgcatggaacagtcacagtggaggtgcagtatgcagggacagatggaccctgcaagatcccagtccagatggcggtggacatgcagaccctgaccccagttggagggctgataaccgccaaccccgtgattactgaaagcactgagaactcaaagatgatgttggagcttgacccaccatttggggattcttacattgtcataggagttggggacaagaaaatcacccaccactggcataggagtggtagcaccatcggaaaggcatttgaggccactgtgagaggcgccaagagaatggcagtcctgggggatacagcctgggacttcggatcagtcgggggtgtgttcaactcactgggtaagggcattcaccagatttttggagcagccttcaaatcactgtttggaggaatgtcctggttctcacagatcctcataggcacgctgctagtgtggttaggtttgaacacaaagaatggatctatctccctcacatgcttggccctggggggagtgatgatcttcctctccacggctgtttctgcttgagcggccgctcgagtctagagggcccgtttaaacccgctgatcagcctcgactgtgccttctagttgccagccatctgttgtttgcccctcccccgtgccttccttgaccctggaaggtgccactcccactgtcctttcctaataaaatgaggaaattgcatcgcattgtctgagtaggtgtcattctattctggggggtggggtggggcaggacagcaagggggaggattgggaagacaatagcaggcatgctggggatgcggtgggctctatggcttctactgggcggttttatggacagcaagcgaaccggaattgccagctggggcgccctctggtaaggtgatatctagacccagctttcttgtacaaagttggcattataagaaagcattgcttatcaatttgttgcaacgaacaggtcactatcagtcaaaataaaatcattatttgccatccagctgcagctctggcccgtgtctcaaaatctctgatgttacattgcacaagataaaaatatatcatcatgaacaataaaactgtctgcttacataaacagtaatacaaggggtgttatgagccatattcaacgggaaacgtcgaggccgcgattaaattccaacatggatgctgatttatatgggtataaatgggctcgcgataatgtcgggcaatcaggtgcgacaatctatcgcttgtatgggaagcccgatgcgccagagttgtttctgaaacatggcaaaggtagcgttgccaatgatgttacagatgagatggtcagactaaactggctgacggaatttatgcctcttccgaccatcaagcattttatccgtactcctgatgatgcatggttactcaccactgcgatccccggaaaaacagcattccaggtattagaagaatatcctgattcaggtgaaaatattgttgatgcgctggcagtgttcctgcgccggttgcattcgattcctgtttgtaattgtccttttaacagcgatcgcgtatttcgtctcgctcaggcgcaatcacgaatgaataacggtttggttgatgcgagtgattttgatgacgagcgtaatggctggcctgttgaacaagtctggaaagaaatgcataaacttttgccattctcaccggattcagtcgtcactcatggtgatttctcacttgataaccttatttttgacgaggggaaattaataggttgtattgatgttggacgagtcggaatcgcagaccgataccaggatcttgccatcctatggaactgcctcggtgagttttctccttcattacagaaacggctttttcaaaaatatggtattgataatcctgatatgaataaattgcagtttcatttgatgctcgatgagtttttctaatcagaattggttaattggttgtaacattattcagattgggccccgttccactgagcgtcagaccccgtagaaaagatcaaaggatcttcttgagatcctttttttctgcgcgtaatctgctgcttgcaaacaaaaaaaccaccgctaccagcggtggtttgtttgccggatcaagagctaccaactctttttccgaaggtaactggcttcagcagagcgcagataccaaatactgttcttctagtgtagccgtagttaggccaccacttcaagaactctgtagcaccgcctacatacctcgctctgctaatcctgttaccagtggctgctgccagtggcgataagtcgtgtcttaccgggttggactcaagacgatagttaccggataaggcgcagcggtcgggctgaacggggggttcgtgcacacagcccagcttggagcgaacgacctacaccgaactgagatacctacagcgtgagctatgagaaagcgccacgcttcccgaagggagaaaggcggacaggtatccggtaagcggcagggtcggaacaggagagcgcacgagggagcttccagggggaaacgcctggtatctttatagtcctgtcgggtttcgccacctctgacttgagcgtcgatttttgtgatgctcgtcaggggggcggagcctatggaaaaacgccagcaacgcggcctttttacggttcctggccttttgctggccttttgctcacatgttctttcctgcgttatcccctgattctgtggataaccgtattaccgctagcatggatctcggggacgtctaactactaagcgagagtagggaactgccaggcatcaaataaaacgaaaggctcagtcggaagactgggcctttcgttttatctgttgtttgtcggtgaacgctctcctgagtaggacaaatccgccgggagcggatttgaacgttgtgaagcaacggcccggagggtggcgggcaggacgcccgccataaactgccaggcatcaaactaagcagaaggccatcctgacggatggcctttttgcgtttctacaaactcttcctgttagttagttacttaagctcgggccccaaataatgattttatt

SEQ ID NO: 21 - protein, 672 aa, Artificial Sequence
  Syntheric polypeptide
AEITRRGSAYYMYLDRSDAGKAISFATTLGVNKCHVQIMDLGHMCDATMSYECPMLDEGVEPDDVDCWCNTTSTWVVYGTCHHKKGEARRSRRAVTLPSHSTRKLQTRSQTWLESREYTKHLIKVENWIFRNPGFALVAVAIAWLLGSSTSQKVIYLVMILLIAPAYSIRCIGVSNRDFVEGMSGGTWVDVVLEHGGCVTVMAQDKPTVDIELVTTTVSNMAEVRSYCYEASISDMASDSRCPTQGEAYLDKQSDTQYVCKRTLVDRGWGNGCKDFGKGSLVTCAKFTCSKKMTGKSIQPENLEYRIMLSVHGSQHSGMIVNDTGYETDENRAKVEVTPNSPRAEATLGGFGSLGLDCEPRTGLDFSDLYYLTMNNKHWLVHKEWFHDIPLPWHAGADTGTPHWNNKEALVEFKDAHAKRQTVVVLGSQEGAVHTALAGALEAEMDGAKGKLFSGHLKCRLKMDKLRLKGVSYSLCTAAFTFTKVPAETLHGTVTVEVQYAGTDGPCKIPVQMAVDMQTLTPVGGLITANPVITESTENSKMMLELDPPFGDSYIVIGVGDKKITHHWHRSGSTIGKAFEATVRGAKRMAVLGDTAWDFGSVGGVFNSLGKGIHQIFGAAFKSLFGGMSWFSQILIGTLLVWLGLNTKNGSISLTCLALGGVMIFLSTAVSA

SEQ ID NO: 22 - DNA, 5334 bp, Artificial Sequence
  Plasmid construct pEBZHu2-3 KD
ctttgtacaaaaaagcaggcttcgaaggagatagaaccaattctctaaggaaatacttaaccatggtcgactggatccggtaccgaattcgtcgactagcccatatatggagttccgcgttacataacttacggtaaatggcccgcctggctgaccgcccaacgacccccgcccattgacgtcaataatgacgtatgttcccatagtaacgccaatagggactttccattgacgtcaatgggtggagtatttacggtaaactgcccacttggcagtacatcaagtgtatcatatgccaagtacgccccctattgacgtcaatgacggtaaatggcccgcctggcattatgcccagtacatgaccttatgggactttcctacttggcagtacatctacgtattagtcatcgctattaccatggtgatgcggttttggcagtacatcaatgggcgtggatagcggtttgactcacggggatttccaagtctccaccccattgacgtcaatgggagtttgttttggcaccaaaatcaacgggactttccaaaatgtcgtaacaactccgccccattgacgcaaatgggcggtaggcgtgtacggtgggaggtctatataagcagagctctctggctaactagagaacccactgcttactggcttatcgaaattaatacgactcactatagggagacccaagctggctagcgtttaaacttaagcttggtaccgccgccgccatgggcaagaggtccgccggctcaatcatgtggctcgcgagcttggcagttgtcatagctggtacaagcgccgtggaagtgaccagaagaggcagcgcctactacatgtacctggaccggaacgatgccggcgaggccatcagctttccaaccaccctgggcatgaacaagtgctacatccagatcatggacctgggccacatgtgcgacgccaccatgagctacgagtgccccatgctggacgagggcgtggaacccgacgatgtggactgctggtgcaacaccaccagcacctgggtggtgtacggcacctgtcaccacaagaagggcgaagccagacggtccagacgggccgtgacactgcctagccacagcaccagaaagctgcagacccggtcccagacctggctggaaagcagagagtacaccaagcacctgatccgggtggaaaactggatcttccggaaccccggctttgccctggccgctgctgctattgcttggctgctgggcagcagcacctcccagaaagtgatctacctcgtgatgatcctgctgatcgcccctgcctacagcatccggtgtatcggcgtgtccaaccgggacttcgtggaaggcatgagcggcggcacatgggtggacatcgtgctggaacacggcggctgcgtgacagtgatggcccaggataagcccaccgtggacattgagctcgtgaccaccaccgtgtccaatatggccgaagtgcggagctactgctacgaggccagcatcagcgacatggccagcgacagcagatgccccacacagggcgaggcttacctggacaagcagtccgacacccagtacgtgtgcaagcggaccctggtggatagaggctggggcaatggctgcaaggattttggcaagggcagcctcgtgacctgcgccaagttcgcctgcagcaagaagatgaccggcaagagcatccagcccgagaacctggaataccggatcatgctgagcgtgcacggcagccagcactccggcatgatcgtgaacgacaccggccacgagacagacgagaaccgggccaaggtggaaatcacccccaacagccctagagccgaggccacactgggcggctttggatctctgggcctggactgcgagcctagaaccggcctggatttcagcgacctgtactacctgaccatgaacaacaagcactggctggtgcacaaagagtggttccacgacatccccctgccctggcatgccggcgctgatacaggcacaccccactggaacaacaaagaggctctggtggagttcaaggacgcccacgccaagaggcagaccgtggtggtgctgggatctcaggaaggcgccgtgcatacagctctggctggcgccctggaagccgaaatggatggcgctaagggcagactgtccagcggccacctgaagtgccggctgaagatggacaagctgcggctgaagggcgtgtcctacagcctgtgtaccgccgccttcaccttcaccaagatccccgccgagacactgcacggcaccgtgactgtggaagtgcagtacgccggcaccgacggcccttgtaaagtgcctgctcagatggccgtggatatgcagaccctgacccctgtgggcaggctgatcaccgccaaccctgtgatcaccgagagcaccgagaacagcaagatgatgctggaactggacccccccttcggcgactcctacatcgtgatcggcgtgggagagaagaagatcacccaccactggcacagaagcggcagcaccatcggcaaagccttcgaagccacagtgcggggagccaagagaatggccgtgctgggagataccgcctgggactttggctctgtgggcggagccctgaactctctgggcaagggaatccaccagatcttcggagccgcctttaagagcctgttcggcggcatgagctggttcagccagatcctgatcggcaccctgctgatgtggctgggcctgaacaccaagaacggcagcatctccctgatgtgcctggctctgggaggcgtgctgatcttcctgagcacagccgtgtctgccgacgtgtgagcggccgctcgagtctagagggcccgtttaaacccgctgatcagcctcgactgtgccttctagttgccagccatctgttgtttgcccctcccccgtgccttccttgaccctggaaggtgccactcccactgtcctttcctaataaaatgaggaaattgcatcgcattgtctgagtaggtgtcattctattctggggggtggggtggggcaggacagcaagggggaggattgggaagacaatagcaggcatgctggggatgcggtgggctctatggcttctactgggcggttttatggacagcaagcgaaccggaattgccagctggggcgccctctggtaaggtgatatctagacccagctttcttgtacaaagttggcattataagaaagcattgcttatcaatttgttgcaacgaacaggtcactatcagtcaaaataaaatcattatttgccatccagctgcagctctggcccgtgtctcaaaatctctgatgttacattgcacaagataaaaatatatcatcatgaacaataaaactgtctgcttacataaacagtaatacaaggggtgttatgagccatattcaacgggaaacgtcgaggccgcgattaaattccaacatggatgctgatttatatgggtataaatgggctcgcgataatgtcgggcaatcaggtgcgacaatctatcgcttgtatgggaagcccgatgcgccagagttgtttctgaaacatggcaaaggtagcgttgccaatgatgttacagatgagatggtcagactaaactggctgacggaatttatgcctcttccgaccatcaagcattttatccgtactcctgatgatgcatggttactcaccactgcgatccccggaaaaacagcattccaggtattagaagaatatcctgattcaggtgaaaatattgttgatgcgctggcagtgttcctgcgccggttgcattcgattcctgtttgtaattgtccttttaacagcgatcgcgtatttcgtctcgctcaggcgcaatcacgaatgaataacggtttggttgatgcgagtgattttgatgacgagcgtaatggctggcctgttgaacaagtctggaaagaaatgcataaacttttgccattctcaccggattcagtcgtcactcatggtgatttctcacttgataaccttatttttgacgaggggaaattaataggttgtattgatgttggacgagtcggaatcgcagaccgataccaggatcttgccatcctatggaactgcctcggtgagttttctccttcattacagaaacggctttttcaaaaatatggtattgataatcctgatatgaataaattgcagtttcatttgatgctcgatgagtttttctaatcagaattggttaattggttgtaacattattcagattgggccccgttccactgagcgtcagaccccgtagaaaagatcaaaggatcttcttgagatcctttttttctgcgcgtaatctgctgcttgcaaacaaaaaaaccaccgctaccagcggtggtttgtttgccggatcaagagctaccaactctttttccgaaggtaactggcttcagcagagcgcagataccaaatactgttcttctagtgtagccgtagttaggccaccacttcaagaactctgtagcaccgcctacatacctcgctctgctaatcctgttaccagtggctgctgccagtggcgataagtcgtgtcttaccgggttggactcaagacgatagttaccggataaggcgcagcggtcgggctgaacggggggttcgtgcacacagcccagcttggagcgaacgacctacaccgaactgagatacctacagcgtgagctatgagaaagcgccacgcttcccgaagggagaaaggcggacaggtatccggtaagcggcagggtcggaacaggagagcgcacgagggagcttccagggggaaacgcctggtatctttatagtcctgtcgggtttcgccacctctgacttgagcgtcgatttttgtgatgctcgtcaggggggcggagcctatggaaaaacgccagcaacgcggcctttttacggttcctggccttttgctggccttttgctcacatgttctttcctgcgttatcccctgattctgtggataaccgtattaccgctagcatggatctcggggacgtctaactactaagcgagagtagggaactgccaggcatcaaataaaacgaaaggctcagtcggaagactgggcctttcgttttatctgttgtttgtcggtgaacgctctcctgagtaggacaaatccgccgggagcggatttgaacgttgtgaagcaacggcccggagggtggcgggcaggacgcccgccataaactgccaggcatcaaactaagcagaaggccatcctgacggatggcctttttgcgtttctacaaactcttcctgttagttagttacttaagctcgggccccaaataatgattttatt

SEQ ID NO: 23 - protein, 674 aa, Artificial Sequence
  Synthetic polypeptide
VEVTRRGSAYYMYLDRNDAGEAISFPTTLGMNKCYIQIMDLGHMCDATMSYECPMLDEGVEPDDVDCWCNTTSTWVVYGTCHHKKGEARRSRRAVTLPSHSTRKLQTRSQTWLESREYTKHLIRVENWIFRNPGFALAAAAIAWLLGSSTSQKVIYLVMILLIAPAYSIRCIGVSNRDFVEGMSGGTWVDIVLEHGGCVTVMAQDKPTVDIELVTTTVSNMAEVRSYCYEASISDMASDSRCPTQGEAYLDKQSDTQYVCKRTLVDRGWGNGCKDFGKGSLVTCAKFACSKKMTGKSIQPENLEYRIMLSVHGSQHSGMIVNDTGHETDENRAKVEITPNSPRAEATLGGFGSLGLDCEPRTGLDFSDLYYLTMNNKHWLVHKEWFHDIPLPWHAGADTGTPHWNNKEALVEFKDAHAKRQTVVVLGSQEGAVHTALAGALEAEMDGAKGRLSSGHLKCRLKMDKLRLKGVSYSLCTAAFTFTKIPAETLHGTVTVEVQYAGTDGPCKVPAQMAVDMQTLTPVGRLITANPVITESTENSKMMLELDPPFGDSYIVIGVGEKKITHHWHRSGSTIGKAFEATVRGAKRMAVLGDTAWDFGSVGGALNSLGKGIHQIFGAAFKSLFGGMSWFSQILIGTLLMWLGLNTKNGSISLMCLALGGVLIFLSTAVSADV

SEQ ID NO: 24 - DNA, 32 bp, Artificial Sequence
  Synthetic oligonucleotide
caatggctgcaaggactttggcaagggcagcc

SEQ ID NO: 25 - DNA, 35 bp, Artificial Sequence
  Synthetic oligonucleotide
caatggctgccgagactttggcaagggcagcctcg

SEQ ID NO: 26 - DNA, 32 bp, Artificial Sequence
  Synthetic oligonucleotide
caatggctgccgacattttggcaagggcagcc

SEQ ID NO: 27 - DNA, 30 bp, Artificial Sequence
  Synthetic oligonucleotide
caatggctgcgaagattttggcaagggcag

SEQ ID NO: 28 - DNA, 31 bp, Artificial Sequence
  Synthetic oligonucleotide
caatggctgcgaacgatttggcaagggcagc

SEQ ID NO: 29 - DNA, 31 bp, Artificial Sequence
  Synthetic oligonucleotide
gaaacggttgtaaggattttggcaaagggag